European Patent Application EP 4 112 633 A1, published January 4, 2023. Title: Fusion Protein of Varicella Zoster Virus and Immunogenic Composition Comprising the Same. Applicant: CELLTRION, INC. The sequence listing filed with the application follows.

SEQUENCE LISTING (5 sequences)

SEQ ID NO: 1 - protein, 546 aa, Artificial Sequence
  VZV_truncated gE
MGTVNKPVVGVLMGFGIITGTLRITNPVRASVLRYDDFHTDEDKLDTNSVYEPYYHSDHAESSWVNRGESSRKAYDHNSPYIWPRNDYDGFLENAHEHHGVYNQGRGIDSGERLMQPTQMSAQEDLGDDTGIHVIPTLNGDDRHKIVNVDQRQYGDVFKGDLNPKPQGQRLIEVSVEENHPFTLRAPIQRIYGVRYTETWSFLPSLTCTGDAAPAIQHICLKHTTCFQDVVVDVDCAENTKEDQLAEISYRFQGKKEADQPWIVVNTSTLFDELELDPPEIEPGVLKVLRTEKQYLGVYIWNMRGSDGTSTYATFLVTWKGDEKTRNPTPAVTPQPRGAEFHMWNYHSHVFSVGDTFSLAMHLQYKIHEAPFDLLLEWLYVPIDPTCQPMRLYSTCLYHPNAPQCLSHMNSGCTFTSPHLAQRVASTVYQNCEHADNYTAYCLGISHMEPSFGLILHDGGTTLKFVDTPESLSGLYVFVVYFNGHVEAVAYTVVSTVDHFVNAIEERGFPPTAGQPPATTKPKEITPVNPGTSPLLRYAAWTGGLA

SEQ ID NO: 2 - protein, 227 aa, Artificial Sequence
  Fc(human IgG1)
DKTHTCPPCPAPELLGGPSVFLFPPKPKDTLMISRTPEVTCVVVDVSHEDPEVKFNWYVDGVEVHNAKTKPREEQYNSTYRVVSVLTVLHQDWLNGKEYKCKVSNKALPAPIEKTISKAKGQPREPQVYTLPPSREEMTKNQVSLTCLVKGFYPSDIAVEWESNGQPENNYKTTPPVLDSDGSFFLYSKLTVDKSRWQQGNVFSCSVMHEALHNHYTQKSLSLSPGK

SEQ ID NO: 3 - protein, 232 aa, Artificial Sequence
  Fc(mouse IgG2a)
PRGPTIKPCPPCKCPAPNLLGGPSVFIFPPKIKDVLMISLSPIVTCVVVDVSEDDPDVQISWFVNNVEVHTAQTQTHREDYNSTLRVVSALPIQHQDWMSGKEFKCKVNNKDLPAPIERTISKPKGSVRAPQVYVLPPPEEEMTKKQVTLTCMVTDFMPEDIYVEWTNNGKTELNYKNTEPVLDSDGSYFMYSKLRVEKKNWVERNSYSCSVVHEGLHNHHTTKSFSRTPGK

SEQ ID NO: 4 - protein, 227 aa, Artificial Sequence
  human IgG1 Fc (mutant)
DKTHTCPPCPAPELLAGPDVFLFPPKPKDTLMISRTPEVTCVVVDVSHEDPEVKFNWYVDGVEVHNAKTKPREEQYNSTYRVVSVLTVLHQDWLNGKEYKCKVSNKALPLPEEKTISKAKGQPREPQVYTLPPSREEMTKNQVSLTCLVKGFYPSDIAVEWESNGQPENNYKTTPPVLDSDGSFFLYSKLTVDKSRWQQGNVFSCSVMHEALHNHYTQKSLSLSPGK

SEQ ID NO: 5 - protein, 232 aa, Artificial Sequence
  mouse IgG2a Fc (mutant)
PRGPTIKPCPPCKCPAPNLLAGPDVFIFPPKIKDVLMISLSPIVTCVVVDVSEDDPDVQISWFVNNVEVHTAQTQTHREDYNSTLRVVSALPIQHQDWMSGKEFKCKVNNKDLPLPEERTISKPKGSVRAPQVYVLPPPEEEMTKKQVTLTCMVTDFMPEDIYVEWTNNGKTELNYKNTEPVLDSDGSYFMYSKLRVEKKNWVERNSYSCSVVHEGLHNHHTTKSFSRTPGK